European Patent Application EP 4 631 525 A2, published October 15, 2025. Title: Combined chimeric antigen receptor targeting CD19 and CD20 and application thereof. Applicant: AbelZeta Inc. The sequence listing filed with the application follows.

SEQUENCE LISTING (39 sequences)

SEQ ID NO: 1 - protein, 122 aa, synthetic construct
  REGION 1..122: note = synthesized
  REGION 1..122: note = misc_feature - Heavy chain sequence of single-chain variable region (VH) derived from Leu16 antibody
EVQLQQSGAELVKPGASVKMSCKASGYTFTSYNMHWVKQTPGQGLEWIGAIYPGNGDTSYNQKFKGKATLTADKSSSTAYMQLSSLTSEDSADYYCARSNYYGSSYWFFDVWGAGTTVTVSS

SEQ ID NO: 2 - protein, 106 aa, synthetic construct
  REGION 1..106: note = synthesized
  REGION 1..106: note = misc_feature - Light chain sequence of single-chain variable region (VL) derived from Leu16 antibody
DIVLTQSPAILSASPGEKVTMTCRASSSVNYMDWYQKKPGSSPKPWIYATSNLASGVPARFSGSGSGTSYSLTISRVEAEDAATYYCQQWSFNPPTFGGGTKLEIK

SEQ ID NO: 3 - protein, 122 aa, synthetic construct
  REGION 1..122: note = synthesized
  REGION 1..122: note = misc_feature - Heavy chain sequence of single-chain variable region (VH) derived from Ofatumumab antibody
EVQLVESGGGLVQPGRSLRLSCAASGFTFNDYAMHWVRQAPGKGLEWVSTISWNSGSIGYADSVKGRFTISRDNAKKSLYLQMNSLRAEDTALYYCAKDIQYGNYYYGMDVWGQGTTVTVSS

SEQ ID NO: 4 - protein, 107 aa, synthetic construct
  REGION 1..107: note = synthesized
  REGION 1..107: note = misc_feature - Light chain sequence of single-chain variable region (VL) derived from Ofatumumab antibody
EIVLTQSPATLSLSPGERATLSCRASQSVSSYLAWYQQKPGQAPRLLIYDASNRATGIPARFSGSGSGTDFTLTISSLEPEDFAVYYCQQRSNWPITFGQGTRLEIK

SEQ ID NO: 5 - protein, 107 aa, synthetic construct
  REGION 1..107: note = synthesized
  REGION 1..107: note = misc_feature - Amino acid sequence of the light chain of single-chain variable region (VL) derived from FMC63 antibody
DIQMTQTTSSLSASLGDRVTISCRASQDISKYLNWYQQKPDGTVKLLIYHTSRLHSGVPSRFSGSGSGTDYSLTISNLEQEDIATYFCQQGNTLPYTFGGGTKLEIT

SEQ ID NO: 6 - protein, 120 aa, synthetic construct
  REGION 1..120: note = synthesized
  REGION 1..120: note = misc_feature - Amino acid sequence of the heavy chain of single-chain variable region (VH) derived from FMC63 antibody
EVKLQESGPGLVAPSQSLSVTCTVSGVSLPDYGVSWIRQPPRKGLEWLGVIWGSETTYYNSALKSRLTIIKDNSKSQVFLKMNSLQTDDTAIYYCAKHYYYGGSYAMDYWGQGTSVTVSS

SEQ ID NO: 7 - protein, 5 aa, synthetic construct
  REGION 1..5: note = synthesized
  REGION 1..5: note = misc_feature - Linker sequences
GGGGS

SEQ ID NO: 8 - protein, 21 aa, synthetic construct
  REGION 1..21: note = synthesized
  REGION 1..21: note = misc_feature - Leader sequence of CD8 antigen
MALPVTALLLPLALLLHAARP

SEQ ID NO: 9 - protein, 229 aa, synthetic construct
  REGION 1..229: note = synthesized
  REGION 1..229: note = misc_feature - IgG4 Hinge-CH2-CH3
ESKYGPPCPPCPAPEFLGGPSVFLFPPKPKDTLMISRTPEVTCVVVDVSQEDPEVQFNWYVDGVEVHNAKTKPREEQFNSTYRVVSVLTVLHQDWLNGKEYKCKVSNKGLPSSIEKTISKAKGQPREPQVYTLPPSQEEMTKNQVSLTCLVKGFYPSDIAVEWESNGQPENNYKTTPPVLDSDGSFFLYSRLTVDKSRWQEGNVFSCSVMHEALHNHYTQKSLSLSLGK

SEQ ID NO: 10 - protein, 24 aa, synthetic construct
  REGION 1..24: note = synthesized
  REGION 1..24: note = misc_feature - CD8 transmembrane region
IYIWAPLAGTCGVLLLSLVITLYC

SEQ ID NO: 11 - protein, 27 aa, synthetic construct
  REGION 1..27: note = synthesized
  REGION 1..27: note = misc_feature - CD28 transmembrane region
FWVLVVVGGVLACYSLLVTVAFIIFWV

SEQ ID NO: 12 - protein, 42 aa, synthetic construct
  REGION 1..42: note = synthesized
  REGION 1..42: note = misc_feature - Co-stimulatory factor signal region derived from 4-1BB
KRGRKKLLYIFKQPFMRPVQTTQEEDGCSCRFPEEEEGGCEL

SEQ ID NO: 13 - protein, 41 aa, synthetic construct
  REGION 1..41: note = synthesized
  REGION 1..41: note = misc_feature - Co-stimulatory factor signal region derived from CD28
RSKRSRLLHSDYMNMTPRRPGPTRKHYQPYAPPRDFAAYRS

SEQ ID NO: 14 - protein, 113 aa, synthetic construct
  REGION 1..113: note = synthesized
  REGION 1..113: note = misc_feature - Signaling region of CD3
RVKFSRSADAPAYQQGQNQLYNELNLGRREEYDVLDKRRGRDPEMGGKPQRRKNPQEGLYNELQKDKMAEAYSEIGMKGERRRGKGHDGLYQGLSTATKDTYDALHMQALPPR

SEQ ID NO: 15 - protein, 710 aa, synthetic construct
  REGION 1..710: note = synthesized
  REGION 1..710: note = misc_feature - Amino acid sequence of TN-LEU-19
METDTLLLWVLLLWVPGSTGDIVLTQSPAILSASPGEKVTMTCRASSSVNYMDWYQKKPGSSPKPWIYATSNLASGVPARFSGSGSGTSYSLTISRVEAEDAATYYCQQWSFNPPTFGGGTKLEIKGSTSGGGSGGGSGGGGSSEVQLQQSGAELVKPGASVKMSCKASGYTFTSYNMHWVKQTPGQGLEWIGAIYPGNGDTSYNQKFKGKATLTADKSSSTAYMQLSSLTSEDSADYYCARSNYYGSSYWFFDVWGAGTTVTVSSGGGGSEVKLQESGPGLVAPSQSLSVTCTVSGVSLPDYGVSWIRQPPRKGLEWLGVIWGSETTYYNSALKSRLTIIKDNSKSQVFLKMNSLQTDDTAIYYCAKHYYYGGSYAMDYWGQGTSVTVSSGSTSGSGKPGSGEGSTKGDIQMTQTTSSLSASLGDRVTISCRASQDISKYLNWYQQKPDGTVKLLIYHTSRLHSGVPSRFSGSGSGTDYSLTISNLEQEDIATYFCQQGNTLPYTFGGGTKLEITESKYGPPCPPCPMFWVLVVVGGVLACYSLLVTVAFIIFWVKRGRKKLLYIFKQPFMRPVQTTQEEDGCSCRFPEEEEGGCELRVKFSRSADAPAYQQGQNQLYNELNLGRREEYDVLDKRRGRDPEMGGKPRRKNPQEGLYNELQKDKMAEAYSEIGMKGERRRGKGHDGLYQGLSTATKDTYDALHMQALPPR

SEQ ID NO: 16 - protein, 712 aa, synthetic construct
  REGION 1..712: note = synthesized
  REGION 1..712: note = misc_feature - Amino acid sequence of TN-OF-19
MALPVTALLLPLALLLHAARPEIVLTQSPATLSLSPGERATLSCRASQSVSSYLAWYQQKPGQAPRLLIYDASNRATGIPARFSGSGSGTDFTLTISSLEPEDFAVYYCQQRSNWPITFGQGTRLEIKGSTSGGGSGGGSGGGGSSEVQLVESGGGLVQPGRSLRLSCAASGFTFNDYAMHWVRQAPGKGLEWVSTISWNSGSIGYADSVKGRFTISRDNAKKSLYLQMNSLRAEDTALYYCAKDIQYGNYYYGMDVWGQGTTVTVSSGGGGSEVKLQESGPGLVAPSQSLSVTCTVSGVSLPDYGVSWIRQPPRKGLEWLGVIWGSETTYYNSALKSRLTIIKDNSKSQVFLKMNSLQTDDTAIYYCAKHYYYGGSYAMDYWGQGTSVTVSSGSTSGSGKPGSGEGSTKGDIQMTQTTSSLSASLGDRVTISCRASQDISKYLNWYQQKPDGTVKLLIYHTSRLHSGVPSRFSGSGSGTDYSLTISNLEQEDIATYFCQQGNTLPYTFGGGTKLEITESKYGPPCPPCPMFWVLVVVGGVLACYSLLVTVAFIIFWVKRGRKKLLYIFKQPFMRPVQTTQEEDGCSCRFPEEEEGGCELRVKFSRSADAPAYQQGQNQLYNELNLGRREEYDVLDKRRGRDPEMGGKPRRKNPQEGLYNELQKDKMAEAYSEIGMKGERRRGKGHDGLYQGLSTATKDTYDALHMQALPPR

SEQ ID NO: 17 - DNA, 2130 bp, synthetic construct
  misc_feature 1..2130: note = synthesized
  misc_feature 1..2130: note = Nucleic acid sequence of TN-LEU-19
  source 1..2130: mol_type = other DNA
atggagacagacacactcctgctatgggtgctgctgctctgggttccaggttccacaggtgacattgtgctgacccaatctccagctatcctgtctgcatctccaggggagaaggtcacaatgacttgcagggccagctcaagtgtaaattacatggactggtaccagaagaagccaggatcctcccccaaaccctggatttatgccacatccaacctggcttctggagtccctgctcgcttcagtggcagtgggtctgggacctcttactctctcacaatcagcagagtggaggctgaagatgctgccacttattactgccagcagtggagttttaatccacccacgttcggaggggggaccaagctggaaataaaaggcagtactagcggtggtggctccgggggcggttccggtgggggcggcagcagcgaggtgcagctgcagcagtctggggctgagctggtgaagcctggggcctcagtgaagatgtcctgcaaggcttctggctacacatttaccagttacaatatgcactgggtaaagcagacacctggacagggcctggaatggattggagctatttatccaggaaatggtgatacttcctacaatcagaagttcaaaggcaaggccacattgactgcagacaaatcctccagcacagcctacatgcagctcagcagcctgacatctgaggactctgcggactattactgtgcaagatctaattattacggtagtagctactggttcttcgatgtctggggcgcagggaccacggtcaccgtctcctcaggaggtggtggatccgaggtgaagctgcaggaaagcggccctggcctggtggcccccagccagagcctgagcgtgacctgcaccgtgagcggcgtgagcctgcccgactacggcgtgagctggatccggcagccccccaggaagggcctggaatggctgggcgtgatctggggcagcgagaccacctactacaacagcgccctgaagagccggctgaccatcatcaaggacaacagcaagagccaggtgttcctgaagatgaacagcctgcagaccgacgacaccgccatctactactgcgccaagcactactactacggcggcagctacgccatggactactggggccagggcaccagcgtgaccgtgagcagcggcagcacctccggcagcggcaagcctggcagcggcgagggcagcaccaagggcgacatccagatgacccagaccacctccagcctgagcgccagcctgggcgaccgggtgaccatcagctgccgggccagccaggacatcagcaagtacctgaactggtatcagcagaagcccgacggcaccgtcaagctgctgatctaccacaccagccggctgcacagcggcgtgcccagccggtttagcggcagcggctccggcaccgactacagcctgaccatctccaacctggaacaggaagatatcgccacctacttttgccagcagggcaacacactgccctacacctttggcggcggaacaaagctggaaatcaccgagagcaagtacggaccgccctgccccccttgccctatgttctgggtgctggtggtggtcggaggcgtgctggcctgctacagcctgctggtcaccgtggccttcatcatcttttgggtgaaacggggcagaaagaaactcctgtatatattcaaacaaccatttatgagaccagtacaaactactcaagaggaagatggctgtagctgccgatttccagaagaagaagaaggaggatgtgaactgcgggtgaagttcagcagaagcgccgacgcccctgcctaccagcagggccagaatcagctgtacaacgagctgaacctgggcagaagggaagagtacgacgtcctggataagcggagaggccgggaccctgagatgggcggcaagcctcggcggaagaacccccaggaaggcctgtataacgaactgcagaaagacaagatggccgaggcctacagcgagatcggcatgaagggcgagcggaggcggggcaagggccacgacggcctgtatcagggcctgtccaccgccaccaaggatacctacgacgccctgcacatgcaggccctgcccccaagg

SEQ ID NO: 18 - DNA, 2136 bp, synthetic construct
  misc_feature 1..2136: note = synthesized
  misc_feature 1..2136: note = Nucleic acid sequence of TN-OF-19
  source 1..2136: mol_type = other DNA
atggccttaccagtgaccgccttgctcctgccgctggccttgctgctccacgccgccaggccggaaattgtgttgacacagtctccagccaccctgtctttgtctccaggggaaagagccaccctctcctgcagggccagtcagagtgttagcagctacttagcctggtaccaacagaaacctggccaggctcccaggctcctcatctatgatgcatccaacagggccactggcatcccagccaggttcagtggcagtgggtctgggacagacttcactctcaccatcagcagcctagagcctgaagattttgcagtttattactgtcagcagcgtagcaactggccgatcaccttcggccaagggacacgactggagattaaaggcagtactagcggtggtggctccgggggcggttccggtgggggcggcagcagcgaagtgcagctggtggagtctgggggaggcttggtacagcctggcaggtccctgagactctcctgtgcagcctctggattcacctttaatgattatgccatgcactgggtccggcaagctccagggaagggcctggagtgggtctcaactattagttggaatagtggttccataggctatgcggactctgtgaagggccgattcaccatctccagagacaacgccaagaagtccctgtatctgcaaatgaacagtctgagagctgaggacacggccttgtattactgtgcaaaagatatacagtacggcaactactactacggtatggacgtctggggccaagggaccacggtcaccgtctcctcaggaggtggtggatccgaggtgaagctgcaggaaagcggccctggcctggtggcccccagccagagcctgagcgtgacctgcaccgtgagcggcgtgagcctgcccgactacggcgtgagctggatccggcagccccccaggaagggcctggaatggctgggcgtgatctggggcagcgagaccacctactacaacagcgccctgaagagccggctgaccatcatcaaggacaacagcaagagccaggtgttcctgaagatgaacagcctgcagaccgacgacaccgccatctactactgcgccaagcactactactacggcggcagctacgccatggactactggggccagggcaccagcgtgaccgtgagcagcggcagcacctccggcagcggcaagcctggcagcggcgagggcagcaccaagggcgacatccagatgacccagaccacctccagcctgagcgccagcctgggcgaccgggtgaccatcagctgccgggccagccaggacatcagcaagtacctgaactggtatcagcagaagcccgacggcaccgtcaagctgctgatctaccacaccagccggctgcacagcggcgtgcccagccggtttagcggcagcggctccggcaccgactacagcctgaccatctccaacctggaacaggaagatatcgccacctacttttgccagcagggcaacacactgccctacacctttggcggcggaacaaagctggaaatcaccgagagcaagtacggaccgccctgccccccttgccctatgttctgggtgctggtggtggtcggaggcgtgctggcctgctacagcctgctggtcaccgtggccttcatcatcttttgggtgaaacggggcagaaagaaactcctgtatatattcaaacaaccatttatgagaccagtacaaactactcaagaggaagatggctgtagctgccgatttccagaagaagaagaaggaggatgtgaactgcgggtgaagttcagcagaagcgccgacgcccctgcctaccagcagggccagaatcagctgtacaacgagctgaacctgggcagaagggaagagtacgacgtcctggataagcggagaggccgggaccctgagatgggcggcaagcctcggcggaagaacccccaggaaggcctgtataacgaactgcagaaagacaagatggccgaggcctacagcgagatcggcatgaagggcgagcggaggcggggcaagggccacgacggcctgtatcagggcctgtccaccgccaccaaggatacctacgacgccctgcacatgcaggccctgcccccaagg

SEQ ID NO: 19 - protein, 15 aa, synthetic construct
  REGION 1..15: note = synthesized
  REGION 1..15: note = misc_feature - Amino acid sequence of flexible linker I
GGGGSGGGGSGGGGS

SEQ ID NO: 20 - DNA, 45 bp, synthetic construct
  misc_feature 1..45: note = synthesized
  misc_feature 1..45: note = Nucleic acid sequence of flexible linker I
  source 1..45: mol_type = other DNA
ggtggcggtggctcgggcggtggtgggtcgggtggcggcggatct

SEQ ID NO: 21 - DNA, 321 bp, synthetic construct
  misc_feature 1..321: note = synthesized
  misc_feature 1..321: note = Nucleotide sequence of the light chain of single-chain variable region (VL) derived from FMC63 antibody
  source 1..321: mol_type = other DNA
gacatccagatgacacagactacatcctccctgtctgcctctctgggagacagagtcaccatcagttgcagggcaagtcaggacattagtaaatatttaaattggtatcagcagaaaccagatggaactgttaaactcctgatctaccatacatcaagattacactcaggagtcccatcaaggttcagtggcagtgggtctggaacagattattctctcaccattagcaacctggagcaagaagatattgccacttacttttgccaacagggtaatacgcttccgtacacgttcggaggggggaccaagctggagatcaca

SEQ ID NO: 22 - DNA, 360 bp, synthetic construct
  misc_feature 1..360: note = synthesized
  misc_feature 1..360: note = Nucleotide sequence of the heavy chain of single-chain variable region (VH) derived from FMC63 antibody
  source 1..360: mol_type = other DNA
gaggtgaaactgcaggagtcaggacctggcctggtggcgccctcacagagcctgtccgtcacatgcactgtctcaggggtctcattacccgactatggtgtaagctggattcgccagcctccacgaaagggtctggagtggctgggagtaatatggggtagtgaaaccacatactataattcagctctcaaatccagactgaccatcatcaaggacaactccaagagccaagttttcttaaaaatgaacagtctgcaaactgatgacacagccatttactactgtgccaaacattattactacggtggtagctatgctatggactactggggccaaggaacctcagtcaccgtctcctca

SEQ ID NO: 23 - protein, 472 aa, synthetic construct
  REGION 1..472: note = synthesized
  REGION 1..472: note = misc_feature - Chimeric antigen receptor
MDIQLTQSPAILSASPGEKVTMTCRASSSLSFMHWYQQKPGSSPKPWIYATSNLASGVPARFSGSGSGTSYSLTISTVEAEDAASYFCHQWSSNPLTFGAGTKLEISSGGGGSGGGGSGDVMGVDSGGGLVQPGGSRKLSCAAPGFTFSSFGMHWVRQAPEKGLEWVAYISSPSSTLHYADRVKGRFTISRDNPKNTLFLQMKLPSLCYGLLGPRDHVHRLLKTRLSNSIMYFSHFVPVFLPAKPTTTPAPRPPTPAPTIASQPLSLRPEACRPAAGGAVHTRGLDFACDIYIWAPLAGTCGVLLLSLVITLYCRSKRGRKKLLYIFKQPFMRPVQTTQEEDGCSCRFPEEEEGGCELEFRVKFSRSADAPAYQQGQNQLYNELNLGRREEYDVLDKRRGRDPEMGGKPRRKNPQEGLYNELQKDKMAEAYSEIGMKGERRRGKGHDGLYQGLSTATKDTYDALHMQALPPR

SEQ ID NO: 24 - protein, 492 aa, synthetic construct
  REGION 1..492: note = synthesized
  REGION 1..492: note = misc_feature - Chimeric antigen receptor
MALPVTALLLPLALLLHAARPDIQLTQSPAILSASPGEKVTMTCRASSSLSFMHWYQQKPGSSPKPWIYATSNLASGVPARFSGSGSGTSYSLTISTVEAEDAASYFCHQWSSNPLTFGAGTKLEISSGGGGSGGGGSGDVMGVDSGGGLVQPGGSRKLSCAAPGFTFSSFGMHWVRQAPEKGLEWVAYISSPSSTLHYADRVKGRFTISRDNPKNTLFLQMKLPSLCYGLLGPRDHVHRLLKTRLSNSIMYFSHFVPVFLPAKPTTTPAPRPPTPAPTIASQPLSLRPEACRPAAGGAVHTRGLDFACDIYIWAPLAGTCGVLLLSLVITLYCRSKRGRKKLLYIFKQPFMRPVQTTQEEDGCSCRFPEEEEGGCELEFRVKFSRSADAPAYQQGQNQLYNELNLGRREEYDVLDKRRGRDPEMGGKPRRKNPQEGLYNELQKDKMAEAYSEIGMKGERRRGKGHDGLYQGLSTATKDTYDALHMQALPPR

SEQ ID NO: 25 - protein, 377 aa, synthetic construct
  REGION 1..377: note = synthesized
  REGION 1..377: note = misc_feature - Chimeric antigen receptor
MALPVTALLLPLALLLHAARPDIQLTQSPAILSASPGEKVTMTCRASSSLSFMHWYQQKPGSSPKPWIYATSNLASGVPARFSGSGSGTSYSLTISTVEAEDAASYFCHQWSSNPLTFGAGTKLEIGGGGSGGGGSGGGGSDVMGVDSGGGLVQPGGSRKLSCAAPGFTFSSFGMHWVRQAPEKGLEWVAYISSPSSTLHYADRVKGRFTISRDNPKNTLFLQMKLPSLCYGLLGPRDHVHRLLTRTTTPAPRPPTPAPTIASQPLSLRPEACRPAAGGAVHTRGLDFACDIYIWAPLAGTCGVLLLSLVITLYCRSKRGRKKLLYIFKQPFMRPVQTTQEEDGCSCRFPEEEEGGCELEFELGTFKTNDLQGSCRS

SEQ ID NO: 26 - protein, 377 aa, synthetic construct
  REGION 1..377: note = synthesized
  REGION 1..377: note = misc_feature - Chimeric antigen receptor
MALPVTALLLPLALLLHAARPDVMGVDSGGGLVQPGGSRKLSCAAPGFTFSSFGMHWVRQAPEKGLEWVAYISSPSSTLHYADRVKGRFTISRDNPKNTLFLQMKLPSLCYGLLGPRDHVHRLLGGGGSGGGGSGGGGSDIQLTQSPAILSASPGEKVTMTCRASSSLSFMHWYQQKPGSSPKPWIYATSNLASGVPARFSGSGSGTSYSLTISTVEAEDAASYFCHQWSSNPLTFGAGTKLEITRTTTPAPRPPTPAPTIASQPLSLRPEACRPAAGGAVHTRGLDFACDIYIWAPLAGTCGVLLLSLVITLYCRSKRGRKKLLYIFKQPFMRPVQTTQEEDGCSCRFPEEEEGGCELEFELGTFKTNDLQGSCRS

SEQ ID NO: 27 - protein, 396 aa, synthetic construct
  REGION 1..396: note = synthesized
  REGION 1..396: note = misc_feature - Chimeric antigen receptor
MALPVTALLLPLALLLHAARPQIVLSQSPAILSASPGEKVTMTCRASSSVSYIHWFQQKPGSSPKPWIYATSNLASGVPVRFSGSGSGTSYSLTISRVEAEDAATYYCQQWTSNPPTFGGGTKLEIKGGGGSGGGGSGGGGSQVQLQQPGAELVKPGASVKMSCKASGYTFTSYNMHWVKQTPGRGLEWIGAIYPGNGDTSYNQKFKGKATLTADKSSSTAYMQLSSLTSEDSAVYYCARSTYYGGDWYFNVWGAGTTVTVSATRTTTPAPRPPTPAPTIASQPLSLRPEACRPAAGGAVHTRGLDFACDIYIWAPLAGTCGVLLLSLVITLYCRSKRGRKKLLYIFKQPFMRPVQTTQEEDGCSCRFPEEEEGGCELEFELGTFKTNDLQGSCRS

SEQ ID NO: 28 - protein, 396 aa, synthetic construct
  REGION 1..396: note = synthesized
  REGION 1..396: note = misc_feature - Chimeric antigen receptor
MALPVTALLLPLALLLHAARPQVQLQQPGAELVKPGASVKMSCKASGYTFTSYNMHWVKQTPGRGLEWIGAIYPGNGDTSYNQKFKGKATLTADKSSSTAYMQLSSLTSEDSAVYYCARSTYYGGDWYFNVWGAGTTVTVSAGGGGSGGGGSGGGGSQIVLSQSPAILSASPGEKVTMTCRASSSVSYIHWFQQKPGSSPKPWIYATSNLASGVPVRFSGSGSGTSYSLTISRVEAEDAATYYCQQWTSNPPTFGGGTKLEIKTRTTTPAPRPPTPAPTIASQPLSLRPEACRPAAGGAVHTRGLDFACDIYIWAPLAGTCGVLLLSLVITLYCRSKRGRKKLLYIFKQPFMRPVQTTQEEDGCSCRFPEEEEGGCELEFELGTFKTNDLQGSCRS

SEQ ID NO: 29 - protein, 715 aa, synthetic construct
  REGION 1..715: note = synthesized
  REGION 1..715: note = misc_feature - Chimeric antigen receptor
MALPVTALLLPLALLLHAARPEVQLQQSGAELVKPGASVKMSCKASGYTFTSYNMHWVKQTPGQGLEWIGAIYPGNGDTSYNQKFKGKATLTADKSSSTAYMQLSSLTSEDSADYYCARSNYYGSSYWFFDVWGAGTTVTVSSGGGGSGGGGSGGGGSDIVLTQSPAILSASPGEKVTMTCRASSSVNYMDWYQKKPGSSPKPWIYATSNLASGVPARFSGSGSGTSYSLTISRVEAEDAATYYCQQWSFNPPTFGGGTKLEIKESKYGPPCPPCPAPEFLGGPSVFLFPPKPKDTLMISRTPEVTCVVVDVSQEDPEVQFNWYVDGVEVHNAKTKPREEQFNSTYRVVSVLTVLHQDWLNGKEYKCKVSNKGLPSSIEKTISKAKGQPREPQVYTLPPSQEEMTKNQVSLTCLVKGFYPSDIAVEWESNGQPENNYKTTPPVLDSDGSFFLYSRLTVDKSRWQEGNVFSCSVMHEALHNHYTQKSLSLSLGKFWVLVVVGGVLACYSLLVTVAFIIFWVRSKRSRLLHSDYMNMTPRRPGPTRKHYQPYAPPRDFAAYRSKRGRKKLLYIFKQPFMRPVQTTQEEDGCSCRFPEEEEGGCELRVKFSRSADAPAYKQGQNQLYNELNLGRREEYDVLDKRRGRDPEMGGKPRRKNPQEGLYNELQKDKMAEAYSEIGMKGERRRGKGHDGLYQGLSTATKDTYDALHMQALPPR

SEQ ID NO: 30 - protein, 715 aa, synthetic construct; identical to SEQ ID NO: 29
  REGION 1..715: note = synthesized
  REGION 1..715: note = misc_feature - Chimeric antigen receptor

SEQ ID NO: 31 - protein, 671 aa, synthetic construct
  REGION 1..671: note = synthesized
  REGION 1..671: note = misc_feature - Chimeric antigen receptor
MALPVTALLLPLALLLHAARPDIVLTQSPAILSASPGEKVTMTCRASSSVNYMDWYQKKPGSSPKPWIYATSNLASGVPARFSGSGSGTSYSLTISRVEAEDAATYYCQQWSFNPPTFGGGTKLEIKGGGGSGGGGSGGGGSEVQLQQSGAELVKPGASVKMSCKASGYTFTSYNMHWVKQTPGQGLEWIGAIYPGNGDTSYNQKFKGKATLTADKSSSTAYMQLSSLTSEDSADYYCARSNYYGSSYWFFDVWGAGTTVTVSSESKYGPPCPPCPAPEFLGGPSVFLFPPKPKDTLMISRTPEVTCVVVDVSQEDPEVQFNWYVDGVEVHNAKTKPREEQFNSTYRVVSVLTVLHQDWLNGKEYKCKVSNKGLPSSIEKTISKAKGQPREPQVYTLPPSQEEMTKNQVSLTCLVKGFYPSDIAVEWESNGQPENNYKTTPPVLDSDGSFFLYSRLTVDKSRWQEGNVFSCSVMHEALHNHYTQKSLSLSLGKIYIWAPLAGTCGVLLLSLVITLYCKRGRKKLLYIFKQPFMRPVQTTQEEDGCSCRFPEEEEGGCELRVKFSRSADAPAYKQGQNQLYNELNLGRREEYDVLDKRRGRDPEMGGKPRRKNPQEGLYNELQKDKMAEAYSEIGMKGERRRGKGHDGLYQGLSTATKDTYDALHMQALPPR

SEQ ID NO: 32 - protein, 671 aa, synthetic construct
  REGION 1..671: note = synthesized
  REGION 1..671: note = misc_feature - Chimeric antigen receptor
MALPVTALLLPLALLLHAARPEVQLQQSGAELVKPGASVKMSCKASGYTFTSYNMHWVKQTPGQGLEWIGAIYPGNGDTSYNQKFKGKATLTADKSSSTAYMQLSSLTSEDSADYYCARSNYYGSSYWFFDVWGAGTTVTVSSGGGGSGGGGSGGGGSDIVLTQSPAILSASPGEKVTMTCRASSSVNYMDWYQKKPGSSPKPWIYATSNLASGVPARFSGSGSGTSYSLTISRVEAEDAATYYCQQWSFNPPTFGGGTKLEIKESKYGPPCPPCPAPEFLGGPSVFLFPPKPKDTLMISRTPEVTCVVVDVSQEDPEVQFNWYVDGVEVHNAKTKPREEQFNSTYRVVSVLTVLHQDWLNGKEYKCKVSNKGLPSSIEKTISKAKGQPREPQVYTLPPSQEEMTKNQVSLTCLVKGFYPSDIAVEWESNGQPENNYKTTPPVLDSDGSFFLYSRLTVDKSRWQEGNVFSCSVMHEALHNHYTQKSLSLSLGKIYIWAPLAGTCGVLLLSLVITLYCKRGRKKLLYIFKQPFMRPVQTTQEEDGCSCRFPEEEEGGCELRVKFSRSADAPAYKQGQNQLYNELNLGRREEYDVLDKRRGRDPEMGGKPRRKNPQEGLYNELQKDKMAEAYSEIGMKGERRRGKGHDGLYQGLSTATKDTYDALHMQALPPR

SEQ ID NO: 33 - protein, 677 aa, synthetic construct
  REGION 1..677: note = synthesized
  REGION 1..677: note = misc_feature - Chimeric antigen receptor
MALPVTALLLPLALLLHAARPQVQLVQSGAEVKKPGSSVKVSCKASGYAFSYSWINWVRQAPGQGLEWMGRIFPGDGDTDYNGKFKGRVTITADKSTSTAYMELSSLRSEDTAVYYCARNVFDGYWLVYWGQGTLVTVSSGGGGSGGGGSGGGGSDIVMTQTPLSLPVTPGEPASISCRSSKSLLHSNGITYLYWYLQKPGQSPQLLIYQMSNLVSGVPDRFSGSGSGTDFTLKISRVEAEDVGVYYCAQNLELPYTFGGGTKVEIKRTVESKYGPPCPPCPAPEFLGGPSVFLFPPKPKDTLMISRTPEVTCVVVDVSQEDPEVQFNWYVDGVEVHNAKTKPREEQFNSTYRVVSVLTVLHQDWLNGKEYKCKVSNKGLPSSIEKTISKAKGQPREPQVYTLPPSQEEMTKNQVSLTCLVKGFYPSDIAVEWESNGQPENNYKTTPPVLDSDGSFFLYSRLTVDKSRWQEGNVFSCSVMHEALHNHYTQKSLSLSLGKIYIWAPLAGTCGVLLLSLVITLYCKRGRKKLLYIFKQPFMRPVQTTQEEDGCSCRFPEEEEGGCELRVKFSRSADAPAYKQGQNQLYNELNLGRREEYDVLDKRRGRDPEMGGKPRRKNPQEGLYNELQKDKMAEAYSEIGMKGERRRGKGHDGLYQGLSTATKDTYDALHMQALPPR

SEQ ID NO: 34 - protein, 672 aa, synthetic construct
  REGION 1..672: note = synthesized
  REGION 1..672: note = misc_feature - Chimeric antigen receptor
MALPVTALLLPLALLLHAARPEVQLVESGGGLVQPGRSLRLSCAASGFTFNDYAMHWVRQAPGKGLEWVSTISWNSGSIGYADSVKGRFTISRDNAKKSLYLQMNSLRAEDTALYYCAKDIQYGNYYYGMDVWGQGTTVTVSSGGGGSGGGGSGGGGSEIVLTQSPATLSLSPGERATLSCRASQSVSSYLAWYQQKPGQAPRLLIYDASNRATGIPARFSGSGSGTDFTLTISSLEPEDFAVYYCQQRSNWPITFGQGTRLEIKESKYGPPCPPCPAPEFLGGPSVFLFPPKPKDTLMISRTPEVTCVVVDVSQEDPEVQFNWYVDGVEVHNAKTKPREEQFNSTYRVVSVLTVLHQDWLNGKEYKCKVSNKGLPSSIEKTISKAKGQPREPQVYTLPPSQEEMTKNQVSLTCLVKGFYPSDIAVEWESNGQPENNYKTTPPVLDSDGSFFLYSRLTVDKSRWQEGNVFSCSVMHEALHNHYTQKSLSLSLGKIYIWAPLAGTCGVLLLSLVITLYCKRGRKKLLYIFKQPFMRPVQTTQEEDGCSCRFPEEEEGGCELRVKFSRSADAPAYKQGQNQLYNELNLGRREEYDVLDKRRGRDPEMGGKPRRKNPQEGLYNELQKDKMAEAYSEIGMKGERRRGKGHDGLYQGLSTATKDTYDALHMQALPPR

SEQ ID NO: 35 - protein, 653 aa, synthetic construct
  REGION 1..653: note = synthesized
  REGION 1..653: note = misc_feature - Chimeric antigen receptor
MALPVTALLLPLALLLHAARPGDVMGVDSGGGLVQPGGSRKLSCAAPGFTFSSFGMHWVRQAPEKGLEWVAYISSPSSTLHYADRVKGRFTISRDNPKNTLFLQMKLPSLCYGLLGPRDHVHRLLKGGGGSGGGGSGGGGSDIQLTQSPAILSASPGEKVTMTCRASSSLSFMHWYQQKPGSSPKPWIYATSNLASGVPARFSGSGSGTSYSLTISTVEAEDAASYFCHQWSSNPLTFGAGTKLEIESKYGPPCPPCPAPEFLGGPSVFLFPPKPKDTLMISRTPEVTCVVVDVSQEDPEVQFNWYVDGVEVHNAKTKPREEQFNSTYRVVSVLTVLHQDWLNGKEYKCKVSNKGLPSSIEKTISKAKGQPREPQVYTLPPSQEEMTKNQVSLTCLVKGFYPSDIAVEWESNGQPENNYKTTPPVLDSDGSFFLYSRLTVDKSRWQEGNVFSCSVMHEALHNHYTQKSLSLSLGKIYIWAPLAGTCGVLLLSLVITLYCKRGRKKLLYIFKQPFMRPVQTTQEEDGCSCRFPEEEEGGCELRVKFSRSADAPAYKQGQNQLYNELNLGRREEYDVLDKRRGRDPEMGGKPRRKNPQEGLYNELQKDKMAEAYSEIGMKGERRRGKGHDGLYQGLSTATKDTYDALHMQALPPR

SEQ ID NO: 36 - protein, 670 aa, synthetic construct
  REGION 1..670: note = synthesized
  REGION 1..670: note = misc_feature - Chimeric antigen receptor
MALPVTALLLPLALLLHAARPQVQLQQPGAELVKPGASVKMSCKASGYTFTSYNMHWVKQTPGRGLEWIGAIYPGNGDTSYNQKFKGKATLTADKSSSTAYMQLSSLTSEDSAVYYCARSTYYGGDWYFNVWGAGTTVTVSAGGGGSGGGGSGGGGSQIVLSQSPAILSASPGEKVTMTCRASSSVSYIHWFQQKPGSSPKPWIYATSNLASGVPVRFSGSGSGTSYSLTISRVEAEDAATYYCQQWTSNPPTFGGGTKLEIKESKYGPPCPPCPAPEFLGGPSVFLFPPKPKDTLMISRTPEVTCVVVDVSQEDPEVQFNWYVDGVEVHNAKTKPREEQFNSTYRVVSVLTVLHQDWLNGKEYKCKVSNKGLPSSIEKTISKAKGQPREPQVYTLPPSQEEMTKNQVSLTCLVKGFYPSDIAVEWESNGQPENNYKTTPPVLDSDGSFFLYSRLTVDKSRWQEGNVFSCSVMHEALHNHYTQKSLSLSLGKIYIWAPLAGTCGVLLLSLVITLYCKRGRKKLLYIFKQPFMRPVQTTQEEDGCSCRFPEEEEGGCELRVKFSRSADAPAYKQGQNQLYNELNLGRREEYDVLDKRRGRDPEMGGKPRRKNPQEGLYNELQKDKMAEAYSEIGMKGERRRGKGHDGLYQGLSTATKDTYDALHMQALPPR

SEQ ID NO: 37 - protein, 715 aa, synthetic construct
  REGION 1..715: note = synthesized
  REGION 1..715: note = misc_feature - Chimeric antigen receptor
MALPVTALLLPLALLLHAARPEVQLQQSGAELVKPGASVKMSCKASGYTFTSYNMHWVKQTPGQGLEWIGAIYPGNGDTSYNQKFKGKATLTADKSSSTAYMQLSSLTSEDSADYYCARSNYYGSSYWFFDVWGAGTTVTVSSGGGGSGGGGSGGGGSDIVLTQSPAILSASPGEKVTMTCRASSSVNYMDWYQKKPGSSPKPWIYATSNLASGVPARFSGSGSGTSYSLTISRVEAEDAATYYCQQWSFNPPTFGGGTKLEIKESKYGPPCPPCPAPEFEGGPSVFLFPPKPKDTLMISRTPEVTCVVVDVSQEDPEVQFNWYVDGVEVHNAKTKPREEQFQSTYRVVSVLTVLHQDWLNGKEYKCKVSNKGLPSSIEKTISKAKGQPREPQVYTLPPSQEEMTKNQVSLTCLVKGFYPSDIAVEWESNGQPENNYKTTPPVLDSDGSFFLYSRLTVDKSRWQEGNVFSCSVMHEALHNHYTQKSLSLSLGKFWVLVVVGGVLACYSLLVTVAFIIFWVRSKRSRLLHSDYMNMTPRRPGPTRKHYQPYAPPRDFAAYRSKRGRKKLLYIFKQPFMRPVQTTQEEDGCSCRFPEEEEGGCELRVKFSRSADAPAYKQGQNQLYNELNLGRREEYDVLDKRRGRDPEMGGKPRRKNPQEGLYNELQKDKMAEAYSEIGMKGERRRGKGHDGLYQGLSTATKDTYDALHMQALPPR

SEQ ID NO: 38 - protein, 660 aa, synthetic construct
  REGION 1..660: note = synthesized
  REGION 1..660: note = misc_feature - Chimeric antigen receptor
MALPVTALLLPLALLLHAARPEVQLQQSGAELVKPGASVKMSCKASGYTFTSYNMHWVKQTPGQGLEWIGAIYPGNGDTSYNQKFKGKATLTADKSSSTAYMQLSSLTSEDSADYYCARSNYYGSSYWFFDVWGAGTTVTVSSGGGGSGGGGSGGGGSDIVLTQSPAILSASPGEKVTMTCRASSSVNYMDWYQKKPGSSPKPWIYATSNLASGVPARFSGSGSGTSYSLTISRVEAEDAATYYCQQWSFNPPTFGGGTKLEIKESKYGPPCPPCPAPEFEGGPSVFLFPPKPKDTLMISRTPEVTCVVVDVSQEDPEVQFNWYVDGVEVHNAKTKPREEQFQSTYRVVSVLTVLHQDWLNGKEYKCKVSNKGLPSSIEKTISKAKGQPREPQVYTLPPSQEEMTKNQVSLTCLVKGFYPSDIAVEWESNGQPENNYKTTPPVLDSDGSFFLYSRLTVDKSRWQEGNVFSCSVMHEALHNHYTQKSLSLSLGKIYIWAPLAGTCGVLLLSLVITLYCKRGRKKLLYIFKQPFMRPVQTTQEEDGCSCRFPEEEEGGCELRVKFSRSADAPAYKQGQNQLYNELNLGRREEYDVLDKRRGRDPEMGGKPRRKNPQEGLYNELQKDKMAEAYSEIGMKGERRRGKGHDGLYQGLSTATKDTY

SEQ ID NO: 39 - protein, 672 aa, synthetic construct
  REGION 1..672: note = synthesized
  REGION 1..672: note = misc_feature - Chimeric antigen receptor
MALPVTALLLPLALLLHAARPEVQLVESGGGLVQPGRSLRLSCAASGFTFNDYAMHWVRQAPGKGLEWVSTISWNSGSIGYADSVKGRFTISRDNAKKSLYLQMNSLRAEDTALYYCAKDIQYGNYYYGMDVWGQGTTVTVSSGGGGSGGGGSGGGGSEIVLTQSPATLSLSPGERATLSCRASQSVSSYLAWYQQKPGQAPRLLIYDASNRATGIPARFSGSGSGTDFTLTISSLEPEDFAVYYCQQRSNWPITFGQGTRLEIKESKYGPPCPPCPAPEFEGGPSVFLFPPKPKDTLMISRTPEVTCVVVDVSQEDPEVQFNWYVDGVEVHNAKTKPREEQFQSTYRVVSVLTVLHQDWLNGKEYKCKVSNKGLPSSIEKTISKAKGQPREPQVYTLPPSQEEMTKNQVSLTCLVKGFYPSDIAVEWESNGQPENNYKTTPPVLDSDGSFFLYSRLTVDKSRWQEGNVFSCSVMHEALHNHYTQKSLSLSLGKIYIWAPLAGTCGVLLLSLVITLYCKRGRKKLLYIFKQPFMRPVQTTQEEDGCSCRFPEEEEGGCELRVKFSRSADAPAYKQGQNQLYNELNLGRREEYDVLDKRRGRDPEMGGKPRRKNPQEGLYNELQKDKMAEAYSEIGMKGERRRGKGHDGLYQGLSTATKDTYDALHMQALPPR